European Patent Application EP 4 382 539 A1, published June 12, 2024. Title: Antibody that binds to a linker in a new binding manner. Applicant: Noile-Immune Biotech Inc. Application WO PCT/JP2022/029582, filed August 2, 2022. The sequence listing filed with the application follows.

SEQUENCE LISTING (196 sequences)

SEQ ID NO: 1 - protein, 11 aa, synthetic construct
  REGION 1..11: note = C-terminal from HCDR3
WGQGTLVTVSS

SEQ ID NO: 2 - protein, 11 aa, synthetic construct
  REGION 1..11: note = C-terminal from HCDR3 (2)
WGQGTLVTVSS

SEQ ID NO: 3 - protein, 11 aa, synthetic construct
  REGION 1..11: note = C-terminal from HCDR3 (3)
WGQGTLVTVSS

SEQ ID NO: 4 - protein, 10 aa, synthetic construct
  REGION 1..10: note = C-terminal from HCDR3 (4)
WGQGTTLTVS

SEQ ID NO: 5 - protein, 16 aa, synthetic construct
  REGION 1..16: note = C-terminal from HCDR3
WGQGTTVTVSSGILGS

SEQ ID NO: 6 - protein, 5 aa, synthetic construct
  REGION 1..5: note = A part of C-terminal from HCDR3
VTVSS

SEQ ID NO: 7 - protein, 10 aa, synthetic construct
  REGION 1..10: note = C-terminal from LCDR3
FGGGTKLEIK

SEQ ID NO: 8 - protein, 11 aa, synthetic construct
  REGION 1..11: note = C-terminal from LCDR3 (2)
FGAGTKLELKR

SEQ ID NO: 9 - protein, 11 aa, synthetic construct
  REGION 1..11: note = C-terminal from LCDR3 (3)
FGGGTQLTVLS

SEQ ID NO: 10 - protein, 5 aa, synthetic construct
  REGION 1..5: note = A part of C-terminal from LCDR3
KLEIK

SEQ ID NO: 11 - protein, 5 aa, synthetic construct
  REGION 1..5: note = A part of C-terminal from LCDR3 (2)
LELKR

SEQ ID NO: 12 - protein, 5 aa, synthetic construct
  REGION 1..5: note = A part of C-terminal from LCDR3 (3)
LTVLS

SEQ ID NO: 13 - protein, 5 aa, synthetic construct
  REGION 1..5: note = A part of linker
GGGGS

SEQ ID NO: 14 - protein, 6 aa, synthetic construct
  REGION 1..6: note = A part of linker (2)
GGGGSG

SEQ ID NO: 15 - protein, 5 aa, synthetic construct
  REGION 1..5: note = A part of linker (3)
SSADD

SEQ ID NO: 16 - protein, 6 aa, synthetic construct
  REGION 1..6: note = A part of linker (4)
SSADDA

SEQ ID NO: 17 - protein, 7 aa, synthetic construct
  REGION 1..7: note = A part of linker (5)
SSADDAK

SEQ ID NO: 18 - protein, 8 aa, synthetic construct
  REGION 1..8: note = A part of linker (6)
SSADDAKK

SEQ ID NO: 19 - protein, 13 aa, synthetic construct
  REGION 1..13: note = An antigen peptide
VTVSSSSADDAKK

SEQ ID NO: 20 - protein, 11 aa, synthetic construct
  REGION 1..11: note = An antigen peptide (2)
VTVSSGGGGSG

SEQ ID NO: 21 - protein, 16 aa, synthetic construct
  REGION 1..16: note = An antigen peptide (3)
GGVTVSSSSADDAKKC

SEQ ID NO: 22 - protein, 14 aa, synthetic construct
  REGION 1..14: note = An antigen peptide (4)
GGVTVSSGGGGSGC

SEQ ID NO: 23 - protein, 12 aa, synthetic construct
  REGION 1..12: note = An antigen peptide (5)
LEIKSSADDAKK

SEQ ID NO: 24 - protein, 10 aa, synthetic construct
  REGION 1..10: note = An antigen peptide (6)
LEIKGGGGSG

SEQ ID NO: 25 - protein, 10 aa, synthetic construct
  REGION 1..10: note = An example of linkers
GGGGSGGGGS

SEQ ID NO: 26 - protein, 15 aa, synthetic construct
  REGION 1..15: note = An example of linkers (2)
GGGGSGGGGSGGGGS

SEQ ID NO: 27 - protein, 20 aa, synthetic construct
  REGION 1..20: note = An example of linkers (3)
GGGGSGGGGSGGGGSGGGGS

SEQ ID NO: 28 - protein, 25 aa, synthetic construct
  REGION 1..25: note = An example of linkers (4)
GGGGSGGGGSGGGGSGGGGSGGGGS

SEQ ID NO: 29 - protein, 25 aa, synthetic construct
  REGION 1..25: note = An example of linkers (5)
SSADDAKKDAAKKDDAKKDDAKKDG

SEQ ID NO: 30 - protein, 10 aa, synthetic construct
  REGION 1..10: note = A part of N-terminal from HCDR1
QVTLKESGPA

SEQ ID NO: 31 - protein, 10 aa, synthetic construct
  REGION 1..10: note = A part of N-terminal from HCDR1 (2)
QVQLVQSGAE

SEQ ID NO: 32 - protein, 10 aa, synthetic construct
  REGION 1..10: note = A part of N-terminal from HCDR1 (3)
EVQLVQSGAE

SEQ ID NO: 33 - protein, 10 aa, synthetic construct
  REGION 1..10: note = A part of N-terminal from HCDR1 (4)
SQVQLKESGP

SEQ ID NO: 34 - protein, 10 aa, synthetic construct
  REGION 1..10: note = A part of N-terminal from HCDR1 (5)
QVQLQQSGPG

SEQ ID NO: 35 - protein, 10 aa, synthetic construct
  REGION 1..10: note = A part of N-terminal from LCDR1 (6)
DIVMTQSPLS

SEQ ID NO: 36 - protein, 10 aa, synthetic construct
  REGION 1..10: note = A part of N-terminal from LCDR1 (7)
DIVMTQSPDS

SEQ ID NO: 37 - protein, 10 aa, synthetic construct
  REGION 1..10: note = A part of N-terminal from LCDR1 (8)
DIQLTQSPSS

SEQ ID NO: 38 - protein, 10 aa, synthetic construct
  REGION 1..10: note = A part of N-terminal from LCDR1 (9)
DIQMTQSPKF

SEQ ID NO: 39 - protein, 10 aa, synthetic construct
  REGION 1..10: note = A part of N-terminal from LCDR1 (10)
QPVLTQSSSL

SEQ ID NO: 40 - protein, 6 aa, synthetic construct
  REGION 1..6: note = A c-terminal part of a linker
SGGGGS

SEQ ID NO: 41 - protein, 5 aa, synthetic construct
  REGION 1..5: note = A c-terminal part of a linker (2)
AKKDG

SEQ ID NO: 42 - protein, 6 aa, synthetic construct
  REGION 1..6: note = A c-terminal part of a linker (3)
DAKKDG

SEQ ID NO: 43 - protein, 7 aa, synthetic construct
  REGION 1..7: note = A c-terminal part of a linker (4)
DDAKKDG

SEQ ID NO: 44 - protein, 8 aa, synthetic construct
  REGION 1..8: note = A c-terminal part of a linker (5)
KDDAKKDG

SEQ ID NO: 45 - skipped

SEQ ID NO: 46 - protein, 5 aa, synthetic construct
  REGION 1..5: note = A part of N-terminal from LCDR1 (2)
DIVMT

SEQ ID NO: 47 - protein, 5 aa, synthetic construct
  REGION 1..5: note = A part of N-terminal from LCDR1 (3)
DIQLT

SEQ ID NO: 48 - protein, 5 aa, synthetic construct
  REGION 1..5: note = A part of N-terminal from LCDR1 (4)
DIQMT

SEQ ID NO: 49 - protein, 5 aa, synthetic construct
  REGION 1..5: note = A part of N-terminal from LCDR1 (5)
QPVLT

SEQ ID NO: 50 - protein, 13 aa, synthetic construct
  REGION 1..13: note = An antigen peptide (7)
KDDAKKDGQVTLK

SEQ ID NO: 51 - protein, 13 aa, synthetic construct
  REGION 1..13: note = An antigen peptide (8)
KDDAKKDGQVQLV

SEQ ID NO: 52 - protein, 13 aa, synthetic construct
  REGION 1..13: note = An antigen peptide (9)
KDDAKKDGEVQLV

SEQ ID NO: 53 - protein, 13 aa, synthetic construct
  REGION 1..13: note = An antigen peptide (10)
KDDAKKDGSQVQL

SEQ ID NO: 54 - protein, 13 aa, synthetic construct
  REGION 1..13: note = An antigen peptide (11)
KDDAKKDGQVQLQ

SEQ ID NO: 55 - protein, 11 aa, synthetic construct
  REGION 1..11: note = An antigen peptide (12)
SGGGGSQVTLK

SEQ ID NO: 56 - protein, 11 aa, synthetic construct
  REGION 1..11: note = An antigen peptide (13)
SGGGGSQVQLV

SEQ ID NO: 57 - protein, 11 aa, synthetic construct
  REGION 1..11: note = An antigen peptide (14)
SGGGGSEVQLV

SEQ ID NO: 58 - protein, 11 aa, synthetic construct
  REGION 1..11: note = An antigen peptide (15)
SGGGGSSQVQL

SEQ ID NO: 59 - protein, 11 aa, synthetic construct
  REGION 1..11: note = An antigen peptide (16)
SGGGGSQVQLQ

SEQ ID NO: 60 - protein, 16 aa, synthetic construct
  REGION 1..16: note = An antigen peptide (17)
GGKDDAKKDGQVTLKC

SEQ ID NO: 61 - protein, 16 aa, synthetic construct
  REGION 1..16: note = An antigen peptide (18)
GGKDDAKKDGQVQLVC

SEQ ID NO: 62 - protein, 16 aa, synthetic construct
  REGION 1..16: note = An antigen peptide (19)
GGAKKDDAKKEVQLVC

SEQ ID NO: 63 - protein, 16 aa, synthetic construct
  REGION 1..16: note = An antigen peptide (20)
GGKDDAKKDGSQVQLC

SEQ ID NO: 64 - protein, 16 aa, synthetic construct
  REGION 1..16: note = An antigen peptide (21)
GGKDDAKKDGQVQLQC

SEQ ID NO: 65 - protein, 14 aa, synthetic construct
  REGION 1..14: note = An antigen peptide (22)
GGSGGGGSQVTLKC

SEQ ID NO: 66 - protein, 14 aa, synthetic construct
  REGION 1..14: note = An antigen peptide (23)
GGSGGGGSQVQLVC

SEQ ID NO: 67 - protein, 14 aa, synthetic construct
  REGION 1..14: note = An antigen peptide (24)
GGSGGGGSEVQLVC

SEQ ID NO: 68 - protein, 14 aa, synthetic construct
  REGION 1..14: note = An antigen peptide (25)
GGSGGGGSSQVQLC

SEQ ID NO: 69 - protein, 14 aa, synthetic construct
  REGION 1..14: note = An antigen peptide (26)
GGSGGGGSQVQLQC

SEQ ID NO: 70 - protein, 15 aa, synthetic construct
  REGION 1..15: note = An antigen peptide (27)
GGLEIKSSADDAKKC

SEQ ID NO: 71 - protein, 13 aa, synthetic construct
  REGION 1..13: note = An antigen peptide (28)
GGLEIKGGGGSGC

SEQ ID NO: 72 - protein, 10 aa, synthetic construct
  REGION 1..10: note = C-terminal ten amino acids in the first region in the CAR in theExamples
FGGGTKLEIK

SEQ ID NO: 73 - protein, 10 aa, synthetic construct
  REGION 1..10: note = C-terminal ten amino acids in the first region in the CAR in theExamples
FGGGTKVEIK

SEQ ID NO: 74 - protein, 10 aa, synthetic construct
  REGION 1..10: note = C-terminal ten amino acids in the first region in the CAR in theExamples
FGGGTKLEIK

SEQ ID NO: 75 - protein, 10 aa, synthetic construct
  REGION 1..10: note = C-terminal ten amino acids in the first region in the CAR in theExamples
GQGTTVTVSS

SEQ ID NO: 76 - protein, 10 aa, synthetic construct
  REGION 1..10: note = C-terminal ten amino acids in the first region in the CAR in theExamples
GQGTLVTVSA

SEQ ID NO: 77 - protein, 10 aa, synthetic construct
  REGION 1..10: note = C-terminal ten amino acids in the first region in the CAR in theExamples
WGQGTTLTVS

SEQ ID NO: 78 - protein, 10 aa, synthetic construct
  REGION 1..10: note = C-terminal ten amino acids in the first region in the CAR in theExamples
GQGTLVTVSS

SEQ ID NO: 79 - protein, 5 aa, synthetic construct
  REGION 1..5: note = A part of C-terminal from HCDR3
TLTVS

SEQ ID NO: 80 - protein, 5 aa, synthetic construct
  REGION 1..5: note = A part of C-terminal from HCDR3
GILGS

SEQ ID NO: 81 - protein, 10 aa, synthetic construct
  REGION 1..10: note = C-terminal from LCDR3
FGGGTKVEIK

SEQ ID NO: 82 - protein, 5 aa, synthetic construct
  REGION 1..5: note = A part of C-terminal from LCDR3
KVEIK

SEQ ID NO: 83 - protein, 13 aa, synthetic construct
  REGION 1..13: note = An antigen peptide
KDDAKKDGDIVMT

SEQ ID NO: 84 - protein, 13 aa, synthetic construct
  REGION 1..13: note = An antigen peptide
KDDAKKDGDIQLT

SEQ ID NO: 85 - protein, 13 aa, synthetic construct
  REGION 1..13: note = An antigen peptide
KDDAKKDGDIQMT

SEQ ID NO: 86 - protein, 13 aa, synthetic construct
  REGION 1..13: note = An antigen peptide
KDDAKKDGQPVLT

SEQ ID NO: 87 - protein, 11 aa, synthetic construct
  REGION 1..11: note = An antigen peptide
SGGGGSDIVMT

SEQ ID NO: 88 - protein, 11 aa, synthetic construct
  REGION 1..11: note = An antigen peptide
SGGGGSDIQLT

SEQ ID NO: 89 - protein, 11 aa, synthetic construct
  REGION 1..11: note = An antigen peptide
SGGGGSDIQMT

SEQ ID NO: 90 - protein, 11 aa, synthetic construct
  REGION 1..11: note = An antigen peptide
SGGGGSQPVLT

SEQ ID NO: 91 - protein, 118 aa, synthetic construct
  REGION 1..118: note = 2D12-B12, VH
EVKLVESGGGLVQPGRSLKLSCAASGFNFNDYWMGWVRQAPGKGLEWIGEIKKDSSIINYIPSLKDKFTISRDNAQNTLYLQMSKLGSEDTAIYYCARGVEYYGYHYWGQGTLVTVSS

SEQ ID NO: 92 - protein, 10 aa, synthetic construct
  REGION 1..10: note = 2D12-B12, HCDR1
GFNFNDYWMG

SEQ ID NO: 93 - protein, 17 aa, synthetic construct
  REGION 1..17: note = 2D12-B12, HCDR2
EIKKDSSIINYIPSLKD

SEQ ID NO: 94 - protein, 9 aa, synthetic construct
  REGION 1..9: note = 2D12-B12, HCDR3
GVEYYGYHY

SEQ ID NO: 95 - protein, 113 aa, synthetic construct
  REGION 1..113: note = 2D12-B12, VL
DIVMTQSPSSLAVSAGETVTINCKSSQSLLYSGNQKNYLAWYQQKPGQSPKLLIYWASTRHSGVPARFIGSGSGSDFTLTISSVQAEDLAIYCCQQYYDIPYTFGAGTKLELK

SEQ ID NO: 96 - protein, 17 aa, synthetic construct
  REGION 1..17: note = 2D12-B12, LCDR1
KSSQSLLYSGNQKNYLA

SEQ ID NO: 97 - protein, 7 aa, synthetic construct
  REGION 1..7: note = 2D12-B12, LCDR2
WASTRHS

SEQ ID NO: 98 - protein, 9 aa, synthetic construct
  REGION 1..9: note = 2D12-B12, LCDR3
QQYYDIPYT

SEQ ID NO: 99 - protein, 118 aa, synthetic construct
  REGION 1..118: note = 3A4-A10-7, VH
QVQLQQSGAALVKPGASVKMSCKASGYTFTDCWVSWVKQSHGKSLEWIGEIHPNSGTTNFNEKFKGKATLTVDKSTSTAYMELSRLTSEDSAIYYCTRAYGGYPFDYWGQGVMVTVSS

SEQ ID NO: 100 - protein, 10 aa, synthetic construct
  REGION 1..10: note = 3A4-A10-7, HCDR1
GYTFTDCWVS

SEQ ID NO: 101 - protein, 17 aa, synthetic construct
  REGION 1..17: note = 3A4-A10-7, HCDR2
EIHPNSGTTNFNEKFKG

SEQ ID NO: 102 - protein, 9 aa, synthetic construct
  REGION 1..9: note = 3A4-A10-7, HCDR3
AYGGYPFDY

SEQ ID NO: 103 - protein, 129 aa, synthetic construct
  REGION 1..129: note = 3A4-A10-7, VL
GAPFAFLHHLTGSCADLVLTQPKSVSTSLESTVKLSCKLNSGNIGRYYMHWYQQHEGRSPTNMIYRDDKRPDGVPDRFSGSIDSSSNSAFLTINNVQTEDEAIYFCHSYDSSINIFGGGTKLTVLGQPK

SEQ ID NO: 104 - protein, 13 aa, synthetic construct
  REGION 1..13: note = 3A4-A10-7, LCDR1
KLNSGNIGRYYMH

SEQ ID NO: 105 - protein, 7 aa, synthetic construct
  REGION 1..7: note = 3A4-A10-7, LCDR2
RDDKRPD

SEQ ID NO: 106 - protein, 9 aa, synthetic construct
  REGION 1..9: note = 3A4-A10-7, LCDR3
HSYDSSINI

SEQ ID NO: 107 - protein, 10 aa, synthetic construct
  REGION 1..10: note = C-terminal from CDR3 in the First Region
FGGGTKVEIK

SEQ ID NO: 108 - protein, 10 aa, synthetic construct
  REGION 1..10: note = C-terminal from CDR3 in the First Region
FGGGTKLEIK

SEQ ID NO: 109 - protein, 10 aa, synthetic construct
  REGION 1..10: note = C-terminal from CDR3 in the First Region
GQGTLVTVSS

SEQ ID NO: 110 - protein, 10 aa, synthetic construct
  REGION 1..10: note = C-terminal from CDR3 in the First Region
GAGTTVTVSS

SEQ ID NO: 111 - protein, 10 aa, synthetic construct
  REGION 1..10: note = C-terminal from CDR3 in the First Region
GQGTLVTVSA

SEQ ID NO: 112 - protein, 10 aa, synthetic construct
  REGION 1..10: note = C-terminal from CDR3 in the First Region
FGGGTKVEIK

SEQ ID NO: 113 - protein, 10 aa, synthetic construct
  REGION 1..10: note = C-terminal from CDR3 in the First Region
FGGGTKLEIK

SEQ ID NO: 114 - protein, 10 aa, synthetic construct
  REGION 1..10: note = C-terminal from CDR3 in the First Region
FGGGTKLEIK

SEQ ID NO: 115 - protein, 10 aa, synthetic construct
  REGION 1..10: note = C-terminal from CDR3 in the First Region
FGGGTKLEIK

SEQ ID NO: 116 - protein, 10 aa, synthetic construct
  REGION 1..10: note = C-terminal from CDR3 in the First Region
FGGGTKVEIK

SEQ ID NO: 117 - protein, 10 aa, synthetic construct
  REGION 1..10: note = C-terminal from CDR3 in the First Region
GQGTLVTVSS

SEQ ID NO: 118 - protein, 15 aa, synthetic construct
  REGION 1..15: note = C-terminal from CDR3 in the First Region
GQGTTVTVSSGILGS

SEQ ID NO: 119 - protein, 10 aa, synthetic construct
  REGION 1..10: note = C-terminal from CDR3 in the First Region
GQGTLVTVSS

SEQ ID NO: 120 - protein, 5 aa, synthetic construct
  REGION 1..5: note = A part of C-terminal from HCDR3
VTVSA

SEQ ID NO: 121 - protein, 115 aa, synthetic construct
  REGION 1..115: note = 3E7-C1 VH aa
QVQMKESGPGLVQPSETLSLTCTVSGFSLTSYGVSWVRQPSGKGPEWMGRLWNDGDTAYNSALKSRLSISRDTSKNQVFLKMNSLQTDDTGTYYCTTMNGYKDYWGQGVMVTVSS

SEQ ID NO: 122 - protein, 127 aa, synthetic construct
  REGION 1..127: note = 3E7-C1 VL aa
AWTSLLLPLLSLYAGSVTSYELIQPPSASVTLGNTVSLTCVGDELPKRYAYWYQQKPDQSIVRVIYEDSKRPSGISDRFSGSSSGTTATLTIRDAQAEDEADYYCHSTYSDDKLRIFGGGTKLTVLG

SEQ ID NO: 123 - protein, 8 aa, synthetic construct
  REGION 1..8: note = HCDR1 of 3E7-C1 predicted by IMGT
GFSLTSYG

SEQ ID NO: 124 - protein, 7 aa, synthetic construct
  REGION 1..7: note = HCDR2 of 3E7-C1 predicted by IMGT
LWNDGDT

SEQ ID NO: 125 - protein, 9 aa, synthetic construct
  REGION 1..9: note = HCDR3 of 3E7-C1 predicted by IMGT
TTMNGYKDY

SEQ ID NO: 126 - protein, 6 aa, synthetic construct
  REGION 1..6: note = LCDR1 of 3E7-C1 predicted by IMGT
ELPKRY

SEQ ID NO: 127 - skipped

SEQ ID NO: 128 - protein, 11 aa, synthetic construct
  REGION 1..11: note = LCDR3 of 3E7-C1 predicted by IMGT
HSTYSDDKLRI

SEQ ID NO: 129 - protein, 6 aa, synthetic construct
  REGION 1..6: note = HCDR1 of 3E7-C1 predicted by Kabat
TSYGVS

SEQ ID NO: 130 - protein, 16 aa, synthetic construct
  REGION 1..16: note = HCDR2 of 3E7-C1 predicted by Kabat
RLWNDGDTAYNSALKS

SEQ ID NO: 131 - protein, 7 aa, synthetic construct
  REGION 1..7: note = HCDR3 of 3E7-C1 predicted by Kabat
MNGYKDY

SEQ ID NO: 132 - protein, 11 aa, synthetic construct
  REGION 1..11: note = LCDR1 of 3E7-C1 predicted by Kabat
VGDELPKRYAY

SEQ ID NO: 133 - protein, 7 aa, synthetic construct
  REGION 1..7: note = LCDR2 of 3E7-C1 predicted by Kabat
EDSKRPS

SEQ ID NO: 134 - protein, 11 aa, synthetic construct
  REGION 1..11: note = LCDR3 of 3E7-C1 predicted by Kabat
HSTYSDDKLRI

SEQ ID NO: 135 - protein, 7 aa, synthetic construct
  REGION 1..7: note = HCDR1 of 3E7-C1 predicted by Chothia
GFSLTSY

SEQ ID NO: 136 - protein, 5 aa, synthetic construct
  REGION 1..5: note = HCDR2 of 3E7-C1 predicted by Chothia
WNDGD

SEQ ID NO: 137 - protein, 7 aa, synthetic construct
  REGION 1..7: note = HCDR3 of 3E7-C1 predicted by Chothia
MNGYKDY

SEQ ID NO: 138 - protein, 11 aa, synthetic construct
  REGION 1..11: note = LCDR1 of 3E7-C1 predicted by Chothia
VGDELPKRYAY

SEQ ID NO: 139 - protein, 7 aa, synthetic construct
  REGION 1..7: note = LCDR2 of 3E7-C1 predicted by Chothia
EDSKRPS

SEQ ID NO: 140 - protein, 11 aa, synthetic construct
  REGION 1..11: note = LCDR3 of 3E7-C1 predicted by Chothia
HSTYSDDKLRI

SEQ ID NO: 141 - protein, 6 aa, synthetic construct
  REGION 1..6: note = HCDR1 of 3E7-C1 predicted by Contact
TSYGVS

SEQ ID NO: 142 - protein, 12 aa, synthetic construct
  REGION 1..12: note = HCDR2 of 3E7-C1 predicted by Contact
WMGRLWNDGDTA

SEQ ID NO: 143 - protein, 8 aa, synthetic construct
  REGION 1..8: note = HCDR3 of 3E7-C1 predicted by Contact
TTMNGYKD

SEQ ID NO: 144 - protein, 7 aa, synthetic construct
  REGION 1..7: note = LCDR1 of 3E7-C1 predicted by Contact
KRYAYWY

SEQ ID NO: 145 - protein, 10 aa, synthetic construct
  REGION 1..10: note = LCDR2 of 3E7-C1 predicted by Contact
RVIYEDSKRP

SEQ ID NO: 146 - protein, 10 aa, synthetic construct
  REGION 1..10: note = LCDR3 of 3E7-C1 predicted by Contact
HSTYSDDKLR

SEQ ID NO: 147 - protein, 10 aa, synthetic construct
  REGION 1..10: note = HCDR1 of 3E7-C1 predicted by AbM
GFSLTSYGVS

SEQ ID NO: 148 - protein, 9 aa, synthetic construct
  REGION 1..9: note = HCDR2 of 3E7-C1 predicted by AbM
RLWNDGDTA

SEQ ID NO: 149 - protein, 7 aa, synthetic construct
  REGION 1..7: note = HCDR3 of 3E7-C1 predicted by AbM
MNGYKDY

SEQ ID NO: 150 - protein, 11 aa, synthetic construct
  REGION 1..11: note = LCDR1 of 3E7-C1 predicted by AbM
VGDELPKRYAY

SEQ ID NO: 151 - protein, 7 aa, synthetic construct
  REGION 1..7: note = LCDR2 of 3E7-C1 predicted by AbM
EDSKRPS

SEQ ID NO: 152 - protein, 11 aa, synthetic construct
  REGION 1..11: note = LCDR3 of 3E7-C1 predicted by AbM
HSTYSDDKLRI

SEQ ID NO: 153 - protein, 115 aa, synthetic construct
  REGION 1..115: note = 4B9-B11 VH aa
QMQLKESGPGLVQPSETLSLTCTVSGFSLTSYSVSWVRQPSGKGPEWMGRMYYDGDTAYNSALKSRLSISRDTSKNQVFLKMNSLQTDDTGTYYCTRSIGAEDYWGQGVMVTVSS

SEQ ID NO: 154 - protein, 127 aa, synthetic construct
  REGION 1..127: note = 4B9-B11 VL aa
AWTSLLLPLLSLYAGSVTSYELIQPPSASVTLGNTVSLTCVGDELPKRYAYWYQQKPDQSIVRVIYEDSKRPSGISDRFSGSSSGTTATLTIRDAQNEDEADYYCHSTYSDDKLRIFGGGTKLTVLG

SEQ ID NO: 155 - protein, 8 aa, synthetic construct
  REGION 1..8: note = HCDR1 of 4B9-B11 predicted by IMGT
GFSLTSYS

SEQ ID NO: 156 - protein, 7 aa, synthetic construct
  REGION 1..7: note = HCDR2 of 4B9-B11 predicted by IMGT
MYYDGDT

SEQ ID NO: 157 - protein, 9 aa, synthetic construct
  REGION 1..9: note = HCDR3 of 4B9-B11 predicted by IMGT
TRSIGAEDY

SEQ ID NO: 158 - protein, 6 aa, synthetic construct
  REGION 1..6: note = LCDR1 of 4B9-B11 predicted by IMGT
ELPKRY

SEQ ID NO: 159 - skipped

SEQ ID NO: 160 - protein, 11 aa, synthetic construct
  REGION 1..11: note = LCDR3 of 4B9-B11 predicted by IMGT
HSTYSDDKLRI

SEQ ID NO: 161 - protein, 6 aa, synthetic construct
  REGION 1..6: note = HCDR1 of 4B9-B11 predicted by Kabat
TSYSVS

SEQ ID NO: 162 - protein, 16 aa, synthetic construct
  REGION 1..16: note = HCDR2 of 4B9-B11 predicted by Kabat
RMYYDGDTAYNSALKS

SEQ ID NO: 163 - protein, 7 aa, synthetic construct
  REGION 1..7: note = HCDR3 of 4B9-B11 predicted by Kabat
SIGAEDY

SEQ ID NO: 164 - protein, 11 aa, synthetic construct
  REGION 1..11: note = LCDR1 of 4B9-B11 predicted by Kabat
VGDELPKRYAY

SEQ ID NO: 165 - protein, 7 aa, synthetic construct
  REGION 1..7: note = LCDR2 of 4B9-B11 predicted by Kabat
EDSKRPS

SEQ ID NO: 166 - protein, 11 aa, synthetic construct
  REGION 1..11: note = LCDR3 of 4B9-B11 predicted by Kabat
HSTYSDDKLRI

SEQ ID NO: 167 - protein, 7 aa, synthetic construct
  REGION 1..7: note = HCDR1 of 4B9-B11 predicted by Chothia
GFSLTSY

SEQ ID NO: 168 - protein, 5 aa, synthetic construct
  REGION 1..5: note = HCDR2 of 4B9-B11 predicted by Chothia
YYDGD

SEQ ID NO: 169 - protein, 7 aa, synthetic construct
  REGION 1..7: note = HCDR3 of 4B9-B11 predicted by Chothia
SIGAEDY

SEQ ID NO: 170 - protein, 11 aa, synthetic construct
  REGION 1..11: note = LCDR1 of 4B9-B11 predicted by Chothia
VGDELPKRYAY

SEQ ID NO: 171 - protein, 7 aa, synthetic construct
  REGION 1..7: note = LCDR2 of 4B9-B11 predicted by Chothia
EDSKRPS

SEQ ID NO: 172 - protein, 11 aa, synthetic construct
  REGION 1..11: note = LCDR3 of 4B9-B11 predicted by Chothia
HSTYSDDKLRI

SEQ ID NO: 173 - protein, 6 aa, synthetic construct
  REGION 1..6: note = HCDR1 of 4B9-B11 predicted by Contact
TSYSVS

SEQ ID NO: 174 - protein, 12 aa, synthetic construct
  REGION 1..12: note = HCDR2 of 4B9-B11 predicted by Contact
WMGRMYYDGDTA

SEQ ID NO: 175 - protein, 8 aa, synthetic construct
  REGION 1..8: note = HCDR3 of 4B9-B11 predicted by Contact
TRSIGAED

SEQ ID NO: 176 - protein, 7 aa, synthetic construct
  REGION 1..7: note = LCDR1 of 4B9-B11 predicted by Contact
KRYAYWY

SEQ ID NO: 177 - protein, 10 aa, synthetic construct
  REGION 1..10: note = LCDR2 of 4B9-B11 predicted by Contact
RVIYEDSKRP

SEQ ID NO: 178 - protein, 10 aa, synthetic construct
  REGION 1..10: note = LCDR3 of 4B9-B11 predicted by Contact
HSTYSDDKLR

SEQ ID NO: 179 - protein, 8 aa, synthetic construct
  REGION 1..8: note = HCDR1 of 4B9-B11 predicted by AbM
GFSLTSYS

SEQ ID NO: 180 - protein, 9 aa, synthetic construct
  REGION 1..9: note = HCDR2 of 4B9-B11 predicted by AbM
RMYYDGDTA

SEQ ID NO: 181 - protein, 7 aa, synthetic construct
  REGION 1..7: note = HCDR3 of 4B9-B11 predicted by AbM
SIGAEDY

SEQ ID NO: 182 - protein, 11 aa, synthetic construct
  REGION 1..11: note = LCDR1 of 4B9-B11 predicted by AbM
VGDELPKRYAY

SEQ ID NO: 183 - protein, 7 aa, synthetic construct
  REGION 1..7: note = LCDR2 of 4B9-B11 predicted by AbM
EDSKRPS

SEQ ID NO: 184 - protein, 11 aa, synthetic construct
  REGION 1..11: note = LCDR3 of 4B9-B11 predicted by AbM
HSTYSDDKLRI

SEQ ID NO: 185 - skipped

SEQ ID NO: 186 - protein, 5 aa, synthetic construct
  REGION 1..5: note = HCDR2 of 3E7-C1 concensus
WNDGD

SEQ ID NO: 187 - protein, 6 aa, synthetic construct
  REGION 1..6: note = HCDR3 of 3E7-C1 concensus
MNGYKD

SEQ ID NO: 188-189 - skipped (2 entries)

SEQ ID NO: 190 - protein, 10 aa, synthetic construct
  REGION 1..10: note = LCDR3 of 3E7-C1 concensus
HSTYSDDKLR

SEQ ID NO: 191 - skipped

SEQ ID NO: 192 - protein, 5 aa, synthetic construct
  REGION 1..5: note = HCDR2 of 4B9-B11 concensus
YYDGD

SEQ ID NO: 193 - protein, 6 aa, synthetic construct
  REGION 1..6: note = HCDR3 of 4B9-B11 concensus
SIGAED

SEQ ID NO: 194-195 - skipped (2 entries)

SEQ ID NO: 196 - protein, 10 aa, synthetic construct
  REGION 1..10: note = LCDR3 of 4B9-B11 concensus
HSTYSDDKLR